European Patent Application EP 4 516 925 A1, published March 5, 2025. Title: Method and Kit for Detecting DNA. Applicant: Hitachi, Ltd. The sequence listing filed with the application follows.

SEQUENCE LISTING (12 sequences)

SEQ ID NO: 1 - DNA, 29 bp, synthetic construct
  misc_feature 1..29: note = synthetic polynucleotide
  source 1..29: mol_type = other DNA
gtcacattttcattatttttattataagg

SEQ ID NO: 2 - DNA, 20 bp, synthetic construct
  misc_feature 1..20: note = synthetic polynucleotide
  source 1..20: mol_type = other DNA
gtcaaggcactcttgcctac

SEQ ID NO: 3 - DNA, 18 bp, synthetic construct
  misc_feature 1..18: note = synthetic polynucleotide
  source 1..18: mol_type = other DNA
ctcgatgtgagtttctgc

SEQ ID NO: 4 - DNA, 20 bp, synthetic construct
  misc_feature 1..20: note = synthetic polynucleotide
  source 1..20: mol_type = other DNA
gggtcctcgcctgtgtacag

SEQ ID NO: 5 - DNA, 20 bp, synthetic construct
  misc_feature 1..20: note = synthetic polynucleotide
  source 1..20: mol_type = other DNA
cctgggagctctgggaattt

SEQ ID NO: 6 - DNA, 17 bp, synthetic construct
  misc_feature 1..17: note = synthetic polynucleotide
  source 1..17: mol_type = other DNA
cacacctttggtcactc

SEQ ID NO: 7 - DNA, 21 bp, synthetic construct
  misc_feature 1..21: note = synthetic polynucleotide
  source 1..21: mol_type = other DNA
gctttggtgagatccattgac

SEQ ID NO: 8 - DNA, 20 bp, synthetic construct
  misc_feature 1..20: note = synthetic polynucleotide
  source 1..20: mol_type = other DNA
tccacctggaacttggtctc

SEQ ID NO: 9 - DNA, 15 bp, synthetic construct
  misc_feature 1..15: note = synthetic polynucleotide
  source 1..15: mol_type = other DNA
ttcgctgccgtgtcc

SEQ ID NO: 10 - DNA, 103 bp, synthetic construct
  misc_feature 1..103: note = synthetic polynucleotide
  source 1..103: mol_type = other DNA
gtatcgtcaaggcactcttgcctacgccaccagctccaactaccacaagtttatattcagtcattttcagcaggccttataataaaaataatgaaaatgtgac

SEQ ID NO: 11 - DNA, 60 bp, synthetic construct
  misc_feature 1..60: note = synthetic polynucleotide
  source 1..60: mol_type = other DNA
cctgggagctctgggaatttggagtgaccaaaggtgtgccctgtacacaggcgaggaccc

SEQ ID NO: 12 - DNA, 96 bp, synthetic construct
  misc_feature 1..96: note = synthetic polynucleotide
  source 1..96: mol_type = other DNA
tccacctggaacttggtctcaaagattccagaagtcaggacacggcagcgaagcaggtcctgaaacaaaattgaggtcaatggatctcaccaaagc